European Patent Application EP 4 368 722 A1, published May 15, 2024. Title: METHOD FOR SECRETORY PRODUCTION OF PROTEIN CONTAINING NONCANONICAL AMINO ACID. Applicant: Ajinomoto Co., Inc. The sequence listing filed with the application follows.

SEQUENCE LISTING (142 sequences)

SEQ ID NO: 1 - DNA, 1458 bp, Corynebacterium glutamicum
  source 1..1458: mol_type = genomic DNA
atggaaaacccttatgtcgctgcgctcgatgacgataaaaaagaagtcggcgcaataaaagaagcagaaaaagaacctgaaataggtcccatcagagctgccggacgagccataccgctgcgcacccgcatcattttgatcgtggtgggtatcgccgggcttggtttgctggtcaacgcgattgctgtttccagcctcatgcgtgaagtttcctatacccgcatggatcaagagctagagacctcgatggggacgtgggcgcataacgttgagctgtttaatttcgatggcgtccgccaagggccacccagcgattattatgtggccaaggtttttcctgatggatccagcattattttcaacgatgcacaatcggcacccaatctagctgaaaccaccatcggtactggtccacacactgtggatgctgctagcggttctgcctccaacactccgtggcgtgtgatggcggaaaagaacggtgacattatcaccgtggtgggtaaaagcatggggcgtgaaacaaacctgctgtaccgattggtgatggtgcagatgatcatcggcgcgctgattctggttgctattttgattacttcactcttcctagtcagacgctcgttgcggccgttgagagaagttgaagagaccgccaccaggattgcgggcggtgatttggatcgacgtgtcccgcagtggccaatgaccacagaagtcggacagctgtcgaatgccctcaatatcatgttggagcagctccaagcctcaattctgaccgcccagcaaaaagaagctcagatgcgccgattcgttggcgacgcctcccacgagctccgcacaccactgacctctgtgaagggcttcaccgagctgtattcatcaggtgcaacagatgatgccaactgggtcatgtccaagatcggtggcgaagcccaacgcatgagtgtgcttgtggaagacctcctgtcactgacgcgtgccgaaggccagcaaatggagaagcaccgcgttgacgtgctggaactcgcattggcagtacgcggatccatgcgagcagcctggccagatcgcaccgtcaacgtgtccaataaagccgagtccattccagttgttgaaggcgacccaacccgcctccaccaagttctcaccaacctggttgccaacggactcaaccacggcggaccggacgcggaagtcagcattgagatcaacaccgatgggcaaaacgtgaggattctcgtggcagacaacggtgtcggaatgtctgaagaagatgcccagcatatcttcgagcgtttctaccgcgccgattcctcccgctcacgcgcatccggcggatcgggcctcggccttgcgatcacgaaatccctggtcgaaggccacggcggcacagtcaccgtcgacagcgtgcaaggcgaaggcacggtgttcacgatcaccttgccggcggtttcttaa

SEQ ID NO: 2 - protein, 485 aa, Corynebacterium glutamicum
MENPYVAALDDDKKEVGAIKEAEKEPEIGPIRAAGRAIPLRTRIILIVVGIAGLGLLVNAIAVSSLMREVSYTRMDQELETSMGTWAHNVELFNFDGVRQGPPSDYYVAKVFPDGSSIIFNDAQSAPNLAETTIGTGPHTVDAASGSASNTPWRVMAEKNGDIITVVGKSMGRETNLLYRLVMVQMIIGALILVAILITSLFLVRRSLRPLREVEETATRIAGGDLDRRVPQWPMTTEVGQLSNALNIMLEQLQASILTAQQKEAQMRRFVGDASHELRTPLTSVKGFTELYSSGATDDANWVMSKIGGEAQRMSVLVEDLLSLTRAEGQQMEKHRVDVLELALAVRGSMRAAWPDRTVNVSNKAESIPVVEGDPTRLHQVLTNLVANGLNHGGPDAEVSIEINTDGQNVRILVADNGVGMSEEDAQHIFERFYRADSSRSRASGGSGLGLAITKSLVEGHGGTVTVDSVQGEGTVFTITLPAVS

SEQ ID NO: 3 - protein, 485 aa, Corynebacterium glutamicum
MENPYVAALDDENQEVGVKKEAEKEPEIGPIRAAGRAIPLRTRIILIVVGIAGLGLLVNAIAVSSLMREVSYTRMDQELETSMGTWAHNVELFNFDGVRQGPPSDYYVAKVFPDGSSIIFNDAQSAPDLAETTIGTGPHTVDAASGSASNTPWRVMAEKNGDIITVVGKSMGRETNLLYRLVMVQMIIGALILVAILITSLFLVRRSLRPLREVEETATRIAGGDLDRRVPQWPMTTEVGQLSNALNIMLEQLQASILTAQQKEAQMRRFVGDASHELRTPLTSVKGFTELYSSGATDDANWVMSKIGGEAQRMSVLVEDLLSLTRAEGQQMEKHRVDVLELALAVRGSMRAAWPDRTVNVSNKAESIPVVKGDPTRLHQVLTNLVANGLNHGGPDAEVSIEINTDGQNVRILVADNGVGMSEEDAQHIFERFYRADSSRSRASGGSGLGLAITKSLVEGHGGTVTVDSVQGEGTVFTITLPAVS

SEQ ID NO: 4 - protein, 485 aa, Corynebacterium glutamicum
MENPYVAALDDENQEVGVKKEAEKEPEIGPIRAAGRAIPLRTRIILIVVGIAGLGLLVNAIAVSSLMREVSYTRMDQELETSMGTWAHNVELFNFDGVRQGPPSDYYVAKVFPDGSSIIFNDAQSAPDLAETTIGTGPHTVDAASGSASNTPWRVMAEKNGDIITVVGKSMGRETNLLYRLVVVQMIIGALILVAILITSLFLVRRSLRPLREVEETATRIAGGDLDRRVPQWPMTTEVGQLSNALNIMLEQLQASILTAQQKEAQMRRFVGDASHELRTPLTSVKGFTELYSSGATDDANWVMSKIGGEAQRMSVLVEDLLSLTRAEGQQMEKHRVDVLELALAVRGSMRAAWPDRTVNVSNKAESIPVVEGDPTRLHQVLTNLVANGLNHGGPDAEVSIEINTDGQNVRILVADNGVGMSEEDAQHIFERFYRADSSRSRASGGSGLGLAITKSLVEGHGGTVTVDSVQGEGTVFTITLPAVS

SEQ ID NO: 5 - protein, 504 aa, Corynebacterium callunae
MENPYVAALDKNSNFGAKDTDSAVSDSTEVSQNNDGIGTPATAEPKVGPIRTAGRAMPLRTRIILLVVGIAGLGLLVNAVAVSSLMREVSYTRMDQDLESAMGTWVRNVELFNFDGVRQGPPSDYYVAKVFPDGSSIIFNDAESAPDLGQTTIGTGPHTVEAAEGSASSTHWRVMAAKNGDVITVVGKSMGRESTLLYRLVVVQMVIGVLILIAILIGSFFLVRRSLKPLREVEETASRIAGGELDRRVPQWPMTTEVGQLANALNIMLEQLQTSIMNAQQKEAQMRRFVGDASHELRTPLTSVKGFTELYSSGATQDADWVLSKIGGEAQRMSVLVEDLLSLTRAEGQQMEKHRVDMLELALAVRGSLKAAWPDRTVNVANRSENIPVVEGDPTRLHQVLTNLVANGLNHGGPEAEVNIQVETADDKVKILVIDNGVGMSKEDAEHIFERFYRADTSRSRASGGSGLGLAITKSLVEGHGGTITVDSELGKGTVFSIILPAAE

SEQ ID NO: 6 - protein, 458 aa, Corynebacterium crenatum
IGPIRAAGRAIPLRTRIILIVVGIAGLGLLVNAIAVSSLMREVSYTRMDQELETSMGTWAHNVELFNFDGVRQGPPSDYYVAKVFPDGSSIIFNDAQSAPDLAETTIGTGPHTVDAASGSASNTPWRVMAEKNGDIITVVGKSMGRETNLLYRLVMVQMIIGALILVAILITSLFLVRRSLRPLREVEETATRIAGGDLDRRVPQWPMTTEVGQLSNALNIMLEQLQASILSAQQKEAQMRRFVGDASHELRTPLTSVKGFTELYSSGATDDANWVMSKIGGEAQRMSVLVEDLLSLTRAEGQQMEKHRVDVLELALAVRGSMRAAWPDRTVNVSNKAASIPVVEGDPTRLHQVLTNLVANGLNHGGPDAEVSIEINTDGQNVRILVADNGVGMSEEDAQHIFERFYRADSSRSRASGGSGLGLAITKSLVEGHGGTVTVDSVQGEGTVFTITLPAVS

SEQ ID NO: 7 - protein, 471 aa, Corynebacterium efficiens
MTAPENPHAQVTPVGRFRQAARGVPLRTRIILLVVGIAGLGLLVNAIAVSSLMREVSYSRMDQELESAMNSWAQTAELFGSITLGPPSDYYVVRIFPDGSHMVFNQSDSAPDLGETTIGIGPHTASAAPGSSSSVPWRVIAISDNGTITVVGKSLAPESMLLYRLVIVQLVIGMLIVVAILLSSLYLVNRSLRPLREVEKTAKSIAGGDLDRRVPQWPMTTEVGQLANALNIMLEQLQASILSAQEKESQMRRFVGDASHELRTPLTSVKGYSELYHSGATRDADWVLSKISGEAQRMSVLVEDLLSLTRAEGQQMEKRPVDVLELSLSVASSMRAAWPERSITVVNKTGSLPVVEGDATRLHQVLTNLVNNGLNHGGPDASVEIEISAEGGSVLVRVVDDGVGMTAEDAQHIFERFYRTDTSRSRASGGSGLGLAITKSLVEGHRGTITVDSEVGEGTVFTITLPSRMED

SEQ ID NO: 8 - DNA, 708 bp, Corynebacterium glutamicum
  source 1..708: mol_type = genomic DNA
atggacaaccagtctgacggacaaatccgcgtactcgtcgttgatgacgagccaaacatcgtcgagctgctcaccgtaagccttaaattccaaggcttcgcagtgatgaccgccaacgatggcaatgaagccctgaagattgctcgtgagttccgtccagacgcatacatcctcgatgtcatgatgccaggaatggacggcttcgagctgctgaccaagctgcgcggcgaaggccttgacagcccagttctgtacctcaccgcaaaggatgccgtggagcaccgcatccacggcctgaccatcggcgctgacgactacgtgaccaagcctttctccctggaagaagtaatcacccgcctgcgcgtgattcttcgtcgcggtggagcagttgaagaagacacctcaacttccctgcagtacgcagacctcaccctcaacgatgaaacccacgaggtcaccaaggctggcgaactgatcgatctttccccaactgaattcaacctcctgcgctacctcatgctcaacgctgaagtggtgctgtccaaggcaaagatcctggataacgtgtggcactacgattttggtggcgacggcaacgtcgtggaatcctacatctcctacctgcgccgcaaggtggacacccaggatccgcagctaattcagactgttcgtggcgttggatatgttctgcgcaccccacgtagctaa

SEQ ID NO: 9 - protein, 235 aa, Corynebacterium glutamicum
MDNQSDGQIRVLVVDDEPNIVELLTVSLKFQGFAVMTANDGNEALKIAREFRPDAYILDVMMPGMDGFELLTKLRGEGLDSPVLYLTAKDAVEHRIHGLTIGADDYVTKPFSLEEVITRLRVILRRGGAVEEDTSTSLQYADLTLNDETHEVTKAGELIDLSPTEFNLLRYLMLNAEVVLSKAKILDNVWHYDFGGDGNVVESYISYLRRKVDTQDPQLIQTVRGVGYVLRTPRS

SEQ ID NO: 10 - DNA, 1500 bp, Corynebacterium glutamicum
  source 1..1500: mol_type = genomic DNA
atgtttaacaaccgtatccgcactgcagctctcgctggtgcaatcgcaatctccaccgcagcttccggcgtagctatcccagcattcgctcaggagaccaacccaaccttcaacatcaacaacggcttcaacgatgctgatggatccaccatccagccagttgagccagttaaccacaccgaggaaaccctccgcgacctgactgactccaccggcgcttacctggaagagttccagtacggcaacgttgaggaaatcgttgaagcatacctgcaggttcaggcttccgcagacggattcgatccttctgagcaggctgcttacgaggctttcgaggctgctcgcgttcgtgcatcccaggagctcgcggcttccgctgagaccatcactaagacccgcgagtccgttgcttacgcactcaaggctgaccgcgaagctaccgcagctttcgaggcttacctcagcgctcttcgtcaggtttcagtcatcaacgatctgatcgctgatgctaacgccaagaacaagactgactttgcagagatcgagctctacgatgttctttacaccgacgccgacatctctggcgatgctccacttcttgctcctgcatacaaggagctgaaggaccttcaggctgaggttgacgcagacttcgagtggttgggcgagttcgcaattgataacaatgaagacaactacgtcattcgtactcacatccctgctgtagaggcactcaaggcagcgatcgattcactggtcgacaccgttgagccacttcgtgcagacgctatcgctaagaacatcgaggctcagaagtctgacgttctggttccccagctcttcctcgagcgtgcaactgcacagcgcgacaccctgcgtgttgtagaggcaatcttctctacctctgctcgttacgttgaactctacgagaacgtcgagaacgttaacgttgagaacaagacccttcgccagcactactcttccctgatccctaacctcttcatcgcagcggttggcaacatcaacgagctcaacaatgcagatcaggctgcacgtgagctcttcctcgattgggacaccgacctcaccaccaacgatgaggacgaagcttactaccaggctaagctcgacttcgctatcgagacctacgcaaagatcctgatcaacggtgaagtttggcaggagccactcgcttacgtccagaacctggatgcaggcgcacgtcaggaagcagctgaccgcgaagcagagcgcgcagctgacgcagcataccgcgctgagcagctccgcatcgctcaggaagcagctgacgctcagaaggctctcgctgaggctcttgctaatgcaggcaacaacgacaacggtggcgacaactcctccgacgacaagggaaccggttcttccgacatcggaacctggggacctttcgcagcaattgcagctatcatcgcagcaatcgcagctatcttcccattcctctccggtatcgttaagttctaa

SEQ ID NO: 11 - protein, 499 aa, Corynebacterium glutamicum
MFNNRIRTAALAGAIAISTAASGVAIPAFAQETNPTFNINNGFNDADGSTIQPVEPVNHTEETLRDLTDSTGAYLEEFQYGNVEEIVEAYLQVQASADGFDPSEQAAYEAFEAARVRASQELAASAETITKTRESVAYALKADREATAAFEAYLSALRQVSVINDLIADANAKNKTDFAEIELYDVLYTDADISGDAPLLAPAYKELKDLQAEVDADFEWLGEFAIDNNEDNYVIRTHIPAVEALKAAIDSLVDTVEPLRADAIAKNIEAQKSDVLVPQLFLERATAQRDTLRVVEAIFSTSARYVELYENVENVNVENKTLRQHYSSLIPNLFIAAVGNINELNNADQAARELFLDWDTDLTTNDEDEAYYQAKLDFAIETYAKILINGEVWQEPLAYVQNLDAGARQEAADREAERAADAAYRAEQLRIAQEAADAQKALAEALANAGNNDNGGDNSSDDKGTGSSDIGTWGPFAAIAAIIAAIAAIFPFLSGIVKF

SEQ ID NO: 12 - DNA, 318 bp, Corynebacterium glutamicum
  source 1..318: mol_type = genomic DNA
atgtccctcggaccatgggaaattggaatcattgtcctgctgatcatcgtgctgttcggcgcgaagaagctgcctgatgcagctcgttccatcggccgttccatgcgcatcttcaagtctgaagtcaaagaaatgaacaaggacggcgataccccagaacaacagcagcagcctcagcagcagattgcgcccaaccagatcgaggctcctcagccaaactttgagcagcactaccagggacagcaggttcagcagcctcagaaccctcagacccctgactaccgtcagaactacgaggatccaaaccgcacctcttaa

SEQ ID NO: 13 - protein, 105 aa, Corynebacterium glutamicum
MSLGPWEIGIIVLLIIVLFGAKKLPDAARSIGRSMRIFKSEVKEMNKDGDTPEQQQQPQQQIAPNQIEAPQPNFEQHYQGQQVQQPQNPQTPDYRQNYEDPNRTS

SEQ ID NO: 14 - DNA, 471 bp, Corynebacterium glutamicum
  source 1..471: mol_type = genomic DNA
atgttttctagcgtgggttggggagagatcttcctcttagtcgttgtgggccttgttgtcatcggcccggaacggttgcctcgtttgatccaggacgcacgcgctgcgctgctcgctgcacgtaccgctatcgacaatgcaaagcagtcgttggacagtgattttggttcggaatttgatgaaatccgaaagccactaacccaggttgcacagtacagccggatgagccccaagacggccatcactaaggcgttatttgataatgattcctcgttcctggatgactttgatccaaagaagatcatggccgaaggaacagaaggcgaagctcagcgcaacaagcaggcagctgacaacaatgcgaatgtggtggaacgtccagctgatggttccaccgcacgcccaacgcaaaacgatccaaaagacggcccgaattactcaggtggcgtctcttggaccgatattatttag

SEQ ID NO: 15 - protein, 156 aa, Corynebacterium glutamicum
MFSSVGWGEIFLLVVVGLVVIGPERLPRLIQDARAALLAARTAIDNAKQSLDSDFGSEFDEIRKPLTQVAQYSRMSPKTAITKALFDNDSSFLDDFDPKKIMAEGTEGEAQRNKQAADNNANVVERPADGSTARPTQNDPKDGPNYSGGVSWTDII

SEQ ID NO: 16 - DNA, 945 bp, Corynebacterium glutamicum
  source 1..945: mol_type = genomic DNA
atgtccattgttgagcacatcaaagagtttcgacgccgacttcttatcgctctggcgggcatcctcgtgggcaccattatcggctttatttggtacgatttctcattttggcagatccccactttgggcgagctgctgagggatccgtactgttctctgcctgctgaatcccgctgggccatgagcgactcagaggaatgtcgactgctcgcaaccggcccgtttgatccattcatgcttcgccttaaagtagcggcgttggtgggtatggttcttggctcacccgtgtggctgagccagctgtggggctttatcaccccaggtttgatgaagaatgagcgccgttacaccgcaatcttcgtcacgattgctgttgtgctgtttgtcggcggtgctgttcttgcgtacttcgtcgttgcatatggtttggagttcctccttaccattggtggagacacccaggcagcggccctgactggtgataagtacttcggattcttgctcgcgttgttggcgattttcggcgtgagcttcgaagttccactggtgatcggcatgctcaacattgtgggtatcttgccttacgatgccattaaagataagcgacgcatgatcatcatgattttgttcgtgttcgctgctttcatgacacccggccaggatcctttcaccatgttggtgttggcgctttcactcaccgttctggtagagcttgccctgcagttctgtcgtttcaacgacaaacgccgggacaagaagcgcccagaatggcttgatggcgatgacctctctgcatcaccactggatacttctgctggtggagaagatgctccaagcccagtcgaaaccccagaggcggtggagccttcgcggatgctgaacccaagtggggaggcgtcgataagctataaacccgggcgcgccgacttcggtgacgtgctctag

SEQ ID NO: 17 - protein, 314 aa, Corynebacterium glutamicum
MSIVEHIKEFRRRLLIALAGILVGTIIGFIWYDFSFWQIPTLGELLRDPYCSLPAESRWAMSDSEECRLLATGPFDPFMLRLKVAALVGMVLGSPVWLSQLWGFITPGLMKNERRYTAIFVTIAVVLFVGGAVLAYFVVAYGLEFLLTIGGDTQAAALTGDKYFGFLLALLAIFGVSFEVPLVIGMLNIVGILPYDAIKDKRRMIIMILFVFAAFMTPGQDPFTMLVLALSLTVLVELALQFCRFNDKRRDKKRPEWLDGDDLSASPLDTSAGGEDAPSPVETPEAVEPSRMLNPSGEASISYKPGRADFGDVL

SEQ ID NO: 18 - protein, 39 aa, Escherichia coli
MNNNDLFQASRRRFLAQLGGLTVAGMLGPSLLTPRRATA

SEQ ID NO: 19 - protein, 27 aa, Escherichia coli
MSLSRRQFIQASGIALCAGAVPLKASA

SEQ ID NO: 20 - protein, 48 aa, Bacillus subtilis
MAYDSRFDEWVQKLKEESFQNNTFDRRKFIQGAGKIAGLSLGLTIAQS

SEQ ID NO: 21 - protein, 34 aa, Bacillus subtilis
MKFVKRRTTALVTTLMLSVTSLFALQPSAKAAEH

SEQ ID NO: 22 - protein, 30 aa, Arthrobacter globiformis
MMNLSRRTLLTTGSAATLAYALGMAGSAQA

SEQ ID NO: 23 - protein, 7 aa, synthetic construct
  REGION 1..7: note = Twin-Arginine Motif
  VARIANT 1: note = X can be any naturally occurring amino acid
  VARIANT 4: note = X can be any naturally occurring amino acid
XRRXFLK

SEQ ID NO: 24 - skipped

SEQ ID NO: 25 - protein, 43 aa, Corynebacterium glutamicum
MRDTAFRSIKAKAQAKRRSLWIAAGAVPTAIALTMSLAPMASA

SEQ ID NO: 26 - protein, 30 aa, Corynebacterium glutamicum
MFNNRIRTAALAGAIAISTAASGVAIPAFA

SEQ ID NO: 27 - protein, 25 aa, Corynebacterium stationis
MKRMKSLAAALTVAGAMLAAPVATA

SEQ ID NO: 28 - protein, 469 aa, Corynebacterium glutamicum
QETNPTFNINNGFNDADGSTIQPVEPVNHTEETLRDLTDSTGAYLEEFQYGNVEEIVEAYLQVQASADGFDPSEQAAYEAFEAARVRASQELAASAETITKTRESVAYALKADREATAAFEAYLSALRQVSVINDLIADANAKNKTDFAEIELYDVLYTDADISGDAPLLAPAYKELKDLQAEVDADFEWLGEFAIDNNEDNYVIRTHIPAVEALKAAIDSLVDTVEPLRADAIAKNIEAQKSDVLVPQLFLERATAQRDTLRVVEAIFSTSARYVELYENVENVNVENKTLRQHYSSLIPNLFIAAVGNINELNNADQAARELFLDWDTDLTTNDEDEAYYQAKLDFAIETYAKILINGEVWQEPLAYVQNLDAGARQEAADREAERAADAAYRAEQLRIAQEAADAQKALAEALANAGNNDNGGDNSSDDKGTGSSDIGTWGPFAAIAAIIAAIAAIFPFLSGIVKF

SEQ ID NO: 29-31 - skipped (3 entries)

SEQ ID NO: 32 - protein, 6 aa, Corynebacterium glutamicum
QETNPT

SEQ ID NO: 33 - protein, 6 aa, Corynebacterium glutamicum
QETGTY

SEQ ID NO: 34 - protein, 6 aa, Corynebacterium glutamicum
QETTVT

SEQ ID NO: 35 - protein, 6 aa, Corynebacterium glutamicum
QETPVT

SEQ ID NO: 36 - protein, 6 aa, Corynebacterium glutamicum
QETAVT

SEQ ID NO: 37 - protein, 4 aa, synthetic construct
  REGION 1..4: note = Factor Xa
IEGR

SEQ ID NO: 38 - protein, 6 aa, synthetic construct
  REGION 1..6: note = ProTEV
ENLYFQ

SEQ ID NO: 39 - DNA, 77 bp, Methanocaldococcus jannaschii
  source 1..77: mol_type = genomic DNA
ccggcggtagttcagcctggtagaacggcggactgtagatccgcatgtcgctggttcaaatccggcccgccggacca

SEQ ID NO: 40 - RNA, 77 nt, Methanocaldococcus jannaschii
  source 1..77: mol_type = tRNA
ccggcggtagttcagcctggtagaacggcggactgtagatccgcatgtcgctggttcaaatccggcccgccggacca

SEQ ID NO: 41 - DNA, 76 bp, Methanocaldococcus jannaschii
  source 1..76: mol_type = genomic DNA
cccgccttagttcagagggcagaacggcggactctaaatccgcatggcacgggttcaaatcccgtaggcgggacca

SEQ ID NO: 42 - RNA, 76 nt, Methanocaldococcus jannaschii
  source 1..76: mol_type = tRNA
cccgccttagttcagagggcagaacggcggactctaaatccgcatggcacgggttcaaatcccgtaggcgggacca

SEQ ID NO: 43 - DNA, 77 bp, Methanocaldococcus jannaschii
  source 1..77: mol_type = genomic DNA
cccgccttagttcagcagggcagaacggcggactctaaatccgcatggcacgggttcaaatcccgtaggcgggacca

SEQ ID NO: 44 - RNA, 77 nt, Methanocaldococcus jannaschii
  source 1..77: mol_type = tRNA
cccgccttagttcagcagggcagaacggcggactctaaatccgcatggcacgggttcaaatcccgtaggcgggacca

SEQ ID NO: 45 - DNA, 72 bp, Methanosarcina barkeri
  source 1..72: mol_type = genomic DNA
gggaacctgatcatgtagatcgaatggactctaaatccgttcagccgggttagattcccggggtttccgcca

SEQ ID NO: 46 - RNA, 72 nt, Methanosarcina barkeri
  source 1..72: mol_type = tRNA
gggaacctgatcatgtagatcgaatggactctaaatccgttcagccgggttagattcccggggtttccgcca

SEQ ID NO: 47 - DNA, 921 bp, Methanocaldococcus jannaschii
  source 1..921: mol_type = genomic DNA
atggacgaatttgaaatgataaagagaaacacatctgaaattatcagcgaggaagagttaagagaggttttaaaaaaagatgaaaaatctgcttacataggttttgaaccaagtggtaaaatacatttagggcattatctccaaataaaaaagatgattgatttacaaaatgctggatttgatataattatattgttggctgatttacacgcctatttaaaccagaaaggagagttggatgagattagaaaaataggagattataacaaaaaagtttttgaagcaatggggttaaaggcaaaatatgtttatggaagtgaattccagcttgataaggattatacactgaatgtctatagattggctttaaaaactaccttaaaaagagcaagaaggagtatggaacttatagcaagagaggatgaaaatccaaaggttgctgaagttatctatccaataatgcaggttaatgatattcattatttaggcgttgatgttgcagttggagggatggagcagagaaaaatacacatgttagcaagggagcttttaccaaaaaaggttgtttgtattcacaaccctgtcttaacgggtttggatggagaaggaaagatgagttcttcaaaagggaattttatagctgttgatgactctccagaagagattagggctaagataaagaaagcatactgcccagctggagttgttgaaggaaatccaataatggagatagctaaatacttccttgaatatcctttaaccataaaaaggccagaaaaatttggtggagatttgacagttaatagctatgaggagttagagagtttatttaaaaataaggaattgcatccaatggatttaaaaaatgctgtagctgaagaacttataaagattttagagccaattagaaagagattataa

SEQ ID NO: 48 - protein, 306 aa, Methanocaldococcus jannaschii
MDEFEMIKRNTSEIISEEELREVLKKDEKSAYIGFEPSGKIHLGHYLQIKKMIDLQNAGFDIIILLADLHAYLNQKGELDEIRKIGDYNKKVFEAMGLKAKYVYGSEFQLDKDYTLNVYRLALKTTLKRARRSMELIAREDENPKVAEVIYPIMQVNDIHYLGVDVAVGGMEQRKIHMLARELLPKKVVCIHNPVLTGLDGEGKMSSSKGNFIAVDDSPEEIRAKIKKAYCPAGVVEGNPIMEIAKYFLEYPLTIKRPEKFGGDLTVNSYEELESLFKNKELHPMDLKNAVAEELIKILEPIRKRL

SEQ ID NO: 49 - DNA, 918 bp, Methanocaldococcus jannaschii
  source 1..918: mol_type = genomic DNA
atggatgaatttgaaatgattaagcgtaacaccagcgaaattatctcggaagaagaactgcgtgaagtcctgaaaaaggatgaaaaatcggccaccatcggctttgaaccgagcggtaaaattcatctgggccactatctgcagatcaaaaagatgattgatctgcaaaacgcaggtttcgacattatcattctgctggcggatctgcatgcctatctgaaccagaaaggtgaactggacgaaatccgtaagatcggcgattacaacaagaaggtgtttgaagcgatgggtctgaaagccaagtatgtttacggctctaacttccaactggataaagactataccctgaatgtttaccgtctggcactgaaaaccacgctgaagcgcgctcgtcgctccatggaactgattgcgcgcgaagacgaaaacccgaaagttgcggaagtcatctatccgattatgcaagtgaatccgctgcactaccaaggcgttgatgtcgctgtgggcggtatggaacagcgtaaaatccatatgctggcgcgcgaactgctgccgaaaaaggtggtttgcattcacaacccggtcctgacgggtctggatggcgaaggtaaaatgagctctagtaagggcaattttatcgccgtggatgacagcccggaagaaatccgtgcaaagattaaaaaggcatactgtccggctggcgtcgtggaaggtaatccgatcatggaaattgccaaatattttctggaatacccgctgaccattaaacgcccggaaaagttcggcggtgacctgacggttaactcctacgaagaactggaatcactgttcaaaaataaggaactgcatccgatggatctgaaaaacgccgtcgccgaagaactgattaaaatcctggaaccgatccgcaaacgcctg

SEQ ID NO: 50 - protein, 306 aa, Methanocaldococcus jannaschii
MDEFEMIKRNTSEIISEEELREVLKKDEKSATIGFEPSGKIHLGHYLQIKKMIDLQNAGFDIIILLADLHAYLNQKGELDEIRKIGDYNKKVFEAMGLKAKYVYGSNFQLDKDYTLNVYRLALKTTLKRARRSMELIAREDENPKVAEVIYPIMQVNPLHYQGVDVAVGGMEQRKIHMLARELLPKKVVCIHNPVLTGLDGEGKMSSSKGNFIAVDDSPEEIRAKIKKAYCPAGVVEGNPIMEIAKYFLEYPLTIKRPEKFGGDLTVNSYEELESLFKNKELHPMDLKNAVAEELIKILEPIRKRL

SEQ ID NO: 51 - DNA, 918 bp, Methanocaldococcus jannaschii
  source 1..918: mol_type = genomic DNA
atggacgaatttgaaatgataaagagaaacacatctgaaattatcagcgaggaagagttaagagaggttttaaaaaaagatgaaaaatctgcttacataggttttgaaccaagtggtaaaatacatttagggcattatctccaaataaaaaagatgattgatttacaaaatgctggatttgatataattatattgttggctgatttagccgcctatttaaaccagaaaggagagttggatgagattagaaaaataggagattataacaaaaaagtttttgaagcaatggggttaaaggcaaaatatgtttatggaagtgaattccagcttgataaggattatacactgaatgtctatagattggctttaaaaactaccttaaaaagagcaagaaggagtatggaacttatagcaagagaggatgaaaatccaaaggttgctgaagttatctatccaataatgcaggttaataccagtcattatttaggcgttgatgttgcagttggagggatggagcagagaaaaatacacatgttagcaagggagcttttaccaaaaaaggttgtttgtattcacaaccctgtcttaacgggtttggatggagaaggaaagatgagttcttcaaaagggaattttatagctgttgatgactctccagaagagattagggctaagataaagaaagcatactgcccagctggagttgttgaaggaaatccaataatggagatagctaaatacttccttgaatatcctttaaccataaaaaggccagaaaaatttggtggagatttgacagttaatagctatgaggagttagagagtttatttaaaaataaggaattgcatccaatgcgtttaaaaaatgctgtagctgaagaacttataaagattttagagccaattagaaagagatta

SEQ ID NO: 52 - protein, 306 aa, Methanocaldococcus jannaschii
MDEFEMIKRNTSEIISEEELREVLKKDEKSAYIGFEPSGKIHLGHYLQIKKMIDLQNAGFDIIILLADLAAYLNQKGELDEIRKIGDYNKKVFEAMGLKAKYVYGSEFQLDKDYTLNVYRLALKTTLKRARRSMELIAREDENPKVAEVIYPIMQVNTSHYLGVDVAVGGMEQRKIHMLARELLPKKVVCIHNPVLTGLDGEGKMSSSKGNFIAVDDSPEEIRAKIKKAYCPAGVVEGNPIMEIAKYFLEYPLTIKRPEKFGGDLTVNSYEELESLFKNKELHPMRLKNAVAEELIKILEPIRKRL

SEQ ID NO: 53 - DNA, 1260 bp, Methanosarcina barkeri
  source 1..1260: mol_type = genomic DNA
atggataaaaaaccattagatgttttaatatctgcgaccgggctcgggatgtccaggactggcacgctccacaaaatcaagcaccacgaggtctcaagaagcaaaatatacattgaaatggcgtgtggagaccatcttgttgtgaataattccaggagttgtagaacagccagagcattcagacatcataagtacagaaaaacctgcaaacgatgtagggtttcggacgaggatatcaataattttctcacaagatcaaccgaaagcaaaaacagtgtgaaagttagggtagtttctgctccaaaggtcaaaaaagctatgccgaaatcagtttcaagggctccgaagcctctggaaaattctgtttctgcaaaggcatcaacgaacacatccagatctgtaccttcgcctgcaaaatcaactccaaattcgtctgttcccgcatcggctcctgctccttcacttacaagaagccagcttgatagggttgaggctctcttaagtccagaggataaaatttctctaaatatggcaaagcctttcagggaacttgagcctgaacttgtgacaagaagaaaaaacgattttcagcggctctataccaatgatagagaagactacctcggtaaactcgaacgtgatattacgaaatttttcgtagaccggggttttctggagataaagtctcctatccttattccggcggaatacgtggagagaatgggtattaataatgatactgaactttcaaaacagatcttccgggtggataaaaatctctgcttgaggccaatgcttgccccgactctttacaactatctgcgaaaactcgataggattttaccaggcccaataaaagttttcgaagtcggaccttgttaccggaaagagtctgacggcaaagagcacctggaagaatttactatggtgaacttctgtcagatgggttcgggatgtactcgggaaaatcttgaagctctcatcaaagagtttctggactatctggaaatcgacttcgaaatcgtaggagattcctgtatggtctatggggatactcttgatataatgcacggggacctggagctttcttcggcagtcgtcgggccagtttctcttgatagagaatggggtattgacaaaccatggataggtgcaggttttggtcttgaacgcttgctcaaggttatgcacggctttaaaaacattaagagagcatcaaggtccgaatcttactataatgggatttcaaccaatctgtaa

SEQ ID NO: 54 - protein, 419 aa, Methanosarcina barkeri
MDKKPLDVLISATGLGMSRTGTLHKIKHHEVSRSKIYIEMACGDHLVVNNSRSCRTARAFRHHKYRKTCKRCRVSDEDINNFLTRSTESKNSVKVRVVSAPKVKKAMPKSVSRAPKPLENSVSAKASTNTSRSVPSPAKSTPNSSVPASAPAPSLTRSQLDRVEALLSPEDKISLNMAKPFRELEPELVTRRKNDFQRLYTNDREDYLGKLERDITKFFVDRGFLEIKSPILIPAEYVERMGINNDTELSKQIFRVDKNLCLRPMLAPTLYNYLRKLDRILPGPIKVFEVGPCYRKESDGKEHLEEFTMVNFCQMGSGCTRENLEALIKEFLDYLEIDFEIVGDSCMVYGDTLDIMHGDLELSSAVVGPVSLDREWGIDKPWIGAGFGLERLLKVMHGFKNIKRASRSESYYNGISTNL

SEQ ID NO: 55 - DNA, 1201 bp, Methanocaldococcus jannaschii
  source 1..1201: mol_type = genomic DNA
gatctactcgttactcaaggcaagctcgagcgggacggtcgaaccagcttcaagcgaccggatgagtatgttacagtagatagcgaggatcccccgccttagttcagagggcagaacggcggactctaaatccgcatggcacgggttcaaatcccgtaggcgggaccactgcagatccttagcgaaagctaaggatttttttttcggcttatttgctcaagctgcagcgatctcgagctcggtaccctaatacgactcactataggggatggacgaatttgaaatggatgaatttgaaatgattaagcgtaacaccagcgaaattatctcggaagaagaactgcgtgaagtcctgaaaaaggatgaaaaatcggccaccatcggctttgaaccgagcggtaaaattcatctgggccactatctgcagatcaaaaagatgattgatctgcaaaacgcaggtttcgacattatcattctgctggcggatctgcatgcctatctgaaccagaaaggtgaactggacgaaatccgtaagatcggcgattacaacaagaaggtgtttgaagcgatgggtctgaaagccaagtatgtttacggctctaacttccaactggataaagactataccctgaatgtttaccgtctggcactgaaaaccacgctgaagcgcgctcgtcgctccatggaactgattgcgcgcgaagacgaaaacccgaaagttgcggaagtcatctatccgattatgcaagtgaatccgctgcactaccaaggcgttgatgtcgctgtgggcggtatggaacagcgtaaaatccatatgctggcgcgcgaactgctgccgaaaaaggtggtttgcattcacaacccggtcctgacgggtctggatggcgaaggtaaaatgagctctagtaagggcaattttatcgccgtggatgacagcccggaagaaatccgtgcaaagattaaaaaggcatactgtccggctggcgtcgtggaaggtaatccgatcatggaaattgccaaatattttctggaatacccgctgaccattaaacgcccggaaaagttcggcggtgacctgacggttaactcctacgaagaactggaatcactgttcaaaaataaggaactgcatccgatggatctgaaaaacgccgtcgccgaagaactgattaaaatcctggaaccgatccgcaaacgcctg

SEQ ID NO: 56 - DNA, 1055 bp, synthetic construct
  source 1..1055: mol_type = other DNA
  misc_feature 1..1055: note = VHH antibody 9g8 DNA cassette
caaattcctgtgaagtagctgatttagtacttttcggaggtgtctattcttaccaaatcgtcaagttgtgggtagagtcacctgaatattaattgcaccgcacgggtgatatatgcttatttgctcaagtagttcgaggttaagtgtattttaggtgaacaaatttcagcttcgggtagaagactttcgatgcgcttcagagcttctattgggaaatctgacaccacttgattaaatagcctacccccgaattgggggattggtcattttttgctgtgaaggtagttttgatgcatatgacctgcgtttataaagaaatgtaaacgtgatcagatcgatataaaagaaacagtttgtactcaggtttgaagcattttctccgattcgcctggcaaaaatctcaattgtcgcttacagtttttctcaacgacaggctgctaagctgctagttcggtggcctagtgagtggcgtttacttggataaaagtaatcccatgtcgtgatcagccattttgggttgtttccatagcaatccaaaggtttcgtctttcgatacctattcaaggagccttatgaaacgcatgaaatcgctggctgcggcgctcaccgtcgctggggccatgctggccgcacctgtggcaacggcagaagtccaactcgtcgaatctggcggtggtctggttcaagcgggcggctccctccgtctctcctgtgcggcgtctggtcgtaccttttcctcctacgctatgggctggttccgccaggcaccaggcaaggaacgcgagttcgtggtcgccatcaactggtcctccggctccacctactacgctgattccgtgaagggccgcttcaccatctcccgcgacaacgcaaagaacaccatgtacctgcagatgaactccctcaagccagaagataccgccgtctactactgcgcagccggctaccagatcaactccggcaactacaacttcaaggattacgagtacgactactggggtcaaggcacccaggtcaccgtgtcttctgcgttggagcaccaccaccaccaccac

SEQ ID NO: 57 - DNA, 390 bp, synthetic construct
  source 1..390: mol_type = other DNA
  misc_feature 1..390: note = VHH antibody 9g8 gene
gaagtccaactcgtcgaatctggcggtggtctggttcaagcgggcggctccctccgtctctcctgtgcggcgtctggtcgtaccttttcctcctacgctatgggctggttccgccaggcaccaggcaaggaacgcgagttcgtggtcgccatcaactggtcctccggctccacctactacgctgattccgtgaagggccgcttcaccatctcccgcgacaacgcaaagaacaccatgtacctgcagatgaactccctcaagccagaagataccgccgtctactactgcgcagccggctaccagatcaactccggcaactacaacttcaaggattacgagtacgactactggggtcaaggcacccaggtcaccgtgtcttctgcgttggag

SEQ ID NO: 58 - protein, 130 aa, synthetic construct
  REGION 1..130: note = VHH antibody 9g8
EVQLVESGGGLVQAGGSLRLSCAASGRTFSSYAMGWFRQAPGKEREFVVAINWSSGSTYYADSVKGRFTISRDNAKNTMYLQMNSLKPEDTAVYYCAAGYQINSGNYNFKDYEYDYWGQGTQVTVSSALE

SEQ ID NO: 59 - DNA, 30 bp, synthetic construct
  source 1..30: mol_type = other DNA
  misc_feature 1..30: note = primer
tcctcctaggctatgggctggttccgccag

SEQ ID NO: 60 - DNA, 35 bp, synthetic construct
  source 1..35: mol_type = other DNA
  misc_feature 1..35: note = primer
catagcctaggaggaaaaggtacgaccagacgccg

SEQ ID NO: 61 - DNA, 31 bp, synthetic construct
  source 1..31: mol_type = other DNA
  misc_feature 1..31: note = primer
ctccacctagtacgctgattccgtgaagggc

SEQ ID NO: 62 - DNA, 29 bp, synthetic construct
  source 1..29: mol_type = other DNA
  misc_feature 1..29: note = primer
cagcgtactaggtggagccggaggaccag

SEQ ID NO: 63 - DNA, 31 bp, synthetic construct
  source 1..31: mol_type = other DNA
  misc_feature 1..31: note = primer
cacctactaggctgattccgtgaagggccgc

SEQ ID NO: 64 - DNA, 33 bp, synthetic construct
  source 1..33: mol_type = other DNA
  misc_feature 1..33: note = primer
gaatcagcctagtaggtggagccggaggaccag

SEQ ID NO: 65 - DNA, 32 bp, synthetic construct
  source 1..32: mol_type = other DNA
  misc_feature 1..32: note = primer
caccatgtagctgcagatgaactccctcaagc

SEQ ID NO: 66 - DNA, 31 bp, synthetic construct
  source 1..31: mol_type = other DNA
  misc_feature 1..31: note = primer
ctgcagctacatggtgttctttgcgttgtcg

SEQ ID NO: 67 - DNA, 24 bp, synthetic construct
  source 1..24: mol_type = other DNA
  misc_feature 1..24: note = primer
gccgtctagtactgcgcagccggc

SEQ ID NO: 68 - DNA, 33 bp, synthetic construct
  source 1..33: mol_type = other DNA
  misc_feature 1..33: note = primer
gcagtactagacggcggtatcttctggcttgag

SEQ ID NO: 69 - DNA, 33 bp, synthetic construct
  source 1..33: mol_type = other DNA
  misc_feature 1..33: note = primer
gtctactagtgcgcagccggctaccagatcaac

SEQ ID NO: 70 - DNA, 32 bp, synthetic construct
  source 1..32: mol_type = other DNA
  misc_feature 1..32: note = primer
ctgcgcactagtagacggcggtatcttctggc

SEQ ID NO: 71 - DNA, 33 bp, synthetic construct
  source 1..33: mol_type = other DNA
  misc_feature 1..33: note = primer
gccggctagcagatcaactccggcaactacaac

SEQ ID NO: 72 - DNA, 31 bp, synthetic construct
  source 1..31: mol_type = other DNA
  misc_feature 1..31: note = primer
gatctgctagccggctgcgcagtagtagacg

SEQ ID NO: 73 - DNA, 34 bp, synthetic construct
  source 1..34: mol_type = other DNA
  misc_feature 1..34: note = primer
cggcaactagaacttcaaggattacgagtacgac

SEQ ID NO: 74 - DNA, 32 bp, synthetic construct
  source 1..32: mol_type = other DNA
  misc_feature 1..32: note = primer
gaagttctagttgccggagttgatctggtagc

SEQ ID NO: 75 - DNA, 34 bp, synthetic construct
  source 1..34: mol_type = other DNA
  misc_feature 1..34: note = primer
caaggattaggagtacgactactggggtcaaggc

SEQ ID NO: 76 - DNA, 34 bp, synthetic construct
  source 1..34: mol_type = other DNA
  misc_feature 1..34: note = primer
gtactcctaatccttgaagttgtagttgccggag

SEQ ID NO: 77 - DNA, 28 bp, synthetic construct
  source 1..28: mol_type = other DNA
  misc_feature 1..28: note = primer
gattacgagtaggactactggggtcaag

SEQ ID NO: 78 - DNA, 34 bp, synthetic construct
  source 1..34: mol_type = other DNA
  misc_feature 1..34: note = primer
gtagtcctactcgtaatccttgaagttgtagttg

SEQ ID NO: 79 - DNA, 24 bp, synthetic construct
  source 1..24: mol_type = other DNA
  misc_feature 1..24: note = primer
gtacgactagtggggtcaaggcac

SEQ ID NO: 80 - DNA, 29 bp, synthetic construct
  source 1..29: mol_type = other DNA
  misc_feature 1..29: note = primer
gaccccactagtcgtactcgtaatccttg

SEQ ID NO: 81 - DNA, 954 bp, Methanocaldococcus jannaschii
  source 1..954: mol_type = genomic DNA
taatacgactcactataggggatggacgaatttgaaatggatgaatttgaaatgattaagcgtaacaccagcgaaattatctcggaagaagaactgcgtgaagtcctgaaaaaggatgaaaaatcggccaccatcggctttgaaccgagcggtaaaattcatctgggccactatctgcagatcaaaaagatgattgatctgcaaaacgcaggtttcgacattatcattctgctggcggatctgcatgcctatctgaaccagaaaggtgaactggacgaaatccgtaagatcggcgattacaacaagaaggtgtttgaagcgatgggtctgaaagccaagtatgtttacggctctaacttccaactggataaagactataccctgaatgtttaccgtctggcactgaaaaccacgctgaagcgcgctcgtcgctccatggaactgattgcgcgcgaagacgaaaacccgaaagttgcggaagtcatctatccgattatgcaagtgaatccgctgcactaccaaggcgttgatgtcgctgtgggcggtatggaacagcgtaaaatccatatgctggcgcgcgaactgctgccgaaaaaggtggtttgcattcacaacccggtcctgacgggtctggatggcgaaggtaaaatgagctctagtaagggcaattttatcgccgtggatgacagcccggaagaaatccgtgcaaagattaaaaaggcatactgtccggctggcgtcgtggaaggtaatccgatcatggaaattgccaaatattttctggaatacccgctgaccattaaacgcccggaaaagttcggcggtgacctgacggttaactcctacgaagaactggaatcactgttcaaaaataaggaactgcatccgatggatctgaaaaacgccgtcgccgaagaactgattaaaatcctggaaccgatccgcaaacgcctg

SEQ ID NO: 82 - DNA, 948 bp, synthetic construct
  source 1..948: mol_type = other DNA
  misc_feature 1..948: note = ZHER2 affibody DNA cassette
caaattcctgtgaagtagctgatttagtacttttcggaggtgtctattcttaccaaatcgtcaagttgtgggtagagtcacctgaatattaattgcaccgcacgggtgatatatgcttatttgctcaagtagttcgaggttaagtgtattttaggtgaacaaatttcagcttcgggtagaagactttcgatgcgcttcagagcttctattgggaaatctgacaccacttgattaaatagcctacccccgaattgggggattggtcattttttgctgtgaaggtagttttgatgcatatgacctgcgtttataaagaaatgtaaacgtgatcagatcgatataaaagaaacagtttgtactcaggtttgaagcattttctccgattcgcctggcaaaaatctcaattgtcgcttacagtttttctcaacgacaggctgctaagctgctagttcggtggcctagtgagtggcgtttacttggataaaagtaatcccatgtcgtgatcagccattttgggttgtttccatagcaatccaaaggtttcgtctttcgatacctattcaaggagccttcgcctctatgttttgtacgtcgaataacagtcccacaacagttccccaaaaggtgcgagcgggaaaaggagaagcaaacatggctcagcgaaaactggcctctgtgatcggtgcagcattggcagcatctgctgtactggttggattaatgacacccgcaacagccatgggctcctctcaccaccaccaccaccaccttcaagtcgacaataagttcaataaagaaatgcgtaatgcctactgggaaatcgctctgctcccaaacctgaacaaccagcagaagcgcgcattcatccgctccctctacgatgacccatcccaatccgcaaatctgctcgctgaagccaaaaaactgaatgatgctcaagccccaaag

SEQ ID NO: 83 - DNA, 180 bp, synthetic construct
  source 1..180: mol_type = other DNA
  misc_feature 1..180: note = ZHER2 affibody gene
cttcaagtcgacaataagttcaataaagaaatgcgtaatgcctactgggaaatcgctctgctcccaaacctgaacaaccagcagaagcgcgcattcatccgctccctctacgatgacccatcccaatccgcaaatctgctcgctgaagccaaaaaactgaatgatgctcaagccccaaag

SEQ ID NO: 84 - protein, 60 aa, synthetic construct
  REGION 1..60: note = ZHER2 affibody
LQVDNKFNKEMRNAYWEIALLPNLNNQQKRAFIRSLYDDPSQSANLLAEAKKLNDAQAPK

SEQ ID NO: 85 - DNA, 35 bp, synthetic construct
  source 1..35: mol_type = other DNA
  misc_feature 1..35: note = primer
caataagtagaataaagaaatgcgtaatgcctact

SEQ ID NO: 86 - DNA, 34 bp, synthetic construct
  source 1..34: mol_type = other DNA
  misc_feature 1..34: note = primer
ctttattctacttattgtcgacttgaaggtggtg

SEQ ID NO: 87 - DNA, 27 bp, synthetic construct
  source 1..27: mol_type = other DNA
  misc_feature 1..27: note = primer
gcctactaggaaatcgctctgctccca

SEQ ID NO: 88 - DNA, 35 bp, synthetic construct
  source 1..35: mol_type = other DNA
  misc_feature 1..35: note = primer
gatttcctagtaggcattacgcatttctttattga

SEQ ID NO: 89 - DNA, 31 bp, synthetic construct
  source 1..31: mol_type = other DNA
  misc_feature 1..31: note = primer
ctgctctagaacctgaacaaccagcagaagc

SEQ ID NO: 90 - DNA, 33 bp, synthetic construct
  source 1..33: mol_type = other DNA
  misc_feature 1..33: note = primer
caggttctagagcagagcgatttcccagtaggc

SEQ ID NO: 91 - DNA, 35 bp, synthetic construct
  source 1..35: mol_type = other DNA
  misc_feature 1..35: note = primer
ctccctctaggatgacccatcccaatccgcaaatc

SEQ ID NO: 92 - DNA, 34 bp, synthetic construct
  source 1..34: mol_type = other DNA
  misc_feature 1..34: note = primer
gtcatcctagagggagcggatgaatgcgcgcttc

SEQ ID NO: 93 - DNA, 1356 bp, synthetic construct
  source 1..1356: mol_type = other DNA
  misc_feature 1..1356: note = mRFP DNA cassette
caaattcctgtgaagtagctgatttagtacttttcggaggtgtctattcttaccaaatcgtcaagttgtgggtagagtcacctgaatattaattgcaccgcacgggtgatatatgcttatttgctcaagtagttcgaggttaagtgtattttaggtgaacaaatttcagcttcgggtagaagactttcgatgcgcttcagagcttctattgggaaatctgacaccacttgattaaatagcctacccccgaattgggggattggtcattttttgctgtgaaggtagttttgatgcatatgacctgcgtttataaagaaatgtaaacgtgatcagatcgatataaaagaaacagtttgtactcaggtttgaagcattttctccgattcgcctggcaaaaatctcaattgtcgcttacagtttttctcaacgacaggctgctaagctgctagttcggtggcctagtgagtggcgtttacttggataaaagtaatcccatgtcgtgatcagccattttgggttgtttccatagcaatccaaaggtttcgtctttcgatacctattcaaggagccttcgcctctatgtttaacaaccgtatccgcactgcagctctcgctggtgcaatcgcaatctccaccgcagcttccggcgtagctatcccagcattcgctcaggagaccaacccaacctcctccgaggacgtcatcaaggagttcatgcgcttcaaggtgcgcatggagggctccgtgaacggccacgagttcgagatcgagggcgagggcgagggccgcccctacgagggcacccagaccgccaagctgaaggtgaccaagggcggccccctgcccttcgcctgggacatcctgtcccctcagttccagtacggctccaaggcctacgtgaagcaccccgccgacatccccgactacttgaagctgtccttccccgagggcttcaagtgggagcgcgtgatgaacttcgaggacggcggcgtggtgaccgtgacccaggactcctccctgcaggacggcgagttcatctacaaggtgaagctgcgcggcaccaacttcccctccgacggccccgtaatgcagaagaagaccatgggctgggaggcctccaccgagcggatgtaccccgaggacggcgccctgaagggcgagatcaagatgaggctgaagctgaaggacggcggccactacgacgccgaggtcaagaccacctacatggccaagaagcccgtgcagctgcccggcgcctacaagaccgacatcaagctggacatcacctcccacaacgaggactacaccatcgtggaacagtacgagcgcgccgagggccgccactccaccggcgcc

SEQ ID NO: 94 - DNA, 669 bp, synthetic construct
  source 1..669: mol_type = other DNA
  misc_feature 1..669: note = mRFP gene
tcctccgaggacgtcatcaaggagttcatgcgcttcaaggtgcgcatggagggctccgtgaacggccacgagttcgagatcgagggcgagggcgagggccgcccctacgagggcacccagaccgccaagctgaaggtgaccaagggcggccccctgcccttcgcctgggacatcctgtcccctcagttccagtacggctccaaggcctacgtgaagcaccccgccgacatccccgactacttgaagctgtccttccccgagggcttcaagtgggagcgcgtgatgaacttcgaggacggcggcgtggtgaccgtgacccaggactcctccctgcaggacggcgagttcatctacaaggtgaagctgcgcggcaccaacttcccctccgacggccccgtaatgcagaagaagaccatgggctgggaggcctccaccgagcggatgtaccccgaggacggcgccctgaagggcgagatcaagatgaggctgaagctgaaggacggcggccactacgacgccgaggtcaagaccacctacatggccaagaagcccgtgcagctgcccggcgcctacaagaccgacatcaagctggacatcacctcccacaacgaggactacaccatcgtggaacagtacgagcgcgccgagggccgccactccaccggcgcc

SEQ ID NO: 95 - protein, 223 aa, synthetic construct
  REGION 1..223: note = mRFP
SSEDVIKEFMRFKVRMEGSVNGHEFEIEGEGEGRPYEGTQTAKLKVTKGGPLPFAWDILSPQFQYGSKAYVKHPADIPDYLKLSFPEGFKWERVMNFEDGGVVTVTQDSSLQDGEFIYKVKLRGTNFPSDGPVMQKKTMGWEASTERMYPEDGALKGEIKMRLKLKDGGHYDAEVKTTYMAKKPVQLPGAYKTDIKLDITSHNEDYTIVEQYERAEGRHSTGA

SEQ ID NO: 96 - DNA, 21 bp, synthetic construct
  source 1..21: mol_type = other DNA
  misc_feature 1..21: note = primer
gcccctaggagggcacccaga

SEQ ID NO: 97 - DNA, 20 bp, synthetic construct
  source 1..20: mol_type = other DNA
  misc_feature 1..20: note = primer
cctcctaggggcggccctcg

SEQ ID NO: 98 - DNA, 27 bp, synthetic construct
  source 1..27: mol_type = other DNA
  misc_feature 1..27: note = primer
cccgactagttgaagctgtccttcccc

SEQ ID NO: 99 - DNA, 27 bp, synthetic construct
  source 1..27: mol_type = other DNA
  misc_feature 1..27: note = primer
cttcaactagtcggggatgtcggcggg

SEQ ID NO: 100 - DNA, 168 bp, Methanocaldococcus jannaschii
  source 1..168: mol_type = genomic DNA
gatctactcgttactcaaggcaagctcgagcgggacggtcgaaccagcttcaagcgaccggatgagtatgttacagtagatagcgaggatcccccgccttagttcagagggcagaacggcggactctaaatccgcatggcacgggttcaaatcccgtaggcgggacca

SEQ ID NO: 101 - DNA, 1677 bp, Methanocaldococcus jannaschii
  source 1..1677: mol_type = genomic DNA
aattcctgtgaattagctgatttagtacttttcggaggtgtctattcttaccaaatcgtcaagttgtgggtagagtcacctgaatattaattgcaccgcacgggtgatatatgcttatttgctcaagtagttcgaggttaagtgtattttaggtgaacaaatttcagcttcgggtagaagactttcgatgcgcttcagagcttctattgggaaatctgacaccacttgattaaatagcctacccccgaattgggggattggtcattttttgctgtgaaggtagttttgatgcatatgacctgcgtttataaagaaatgtaaacgtgatcagatcgatataaaagaaacagtttgtactcaggtttgaagcattttctccgattcgcctggcaaaaatctcaattgtcgcttacagtttttctcaacgacaggctgctaagctgctagttcggtggcctagtgagtggcgtttacttggataaaagtaatcccatgtcgtgatcagccattttgggttgtttccatagcaatccaaaggtttcgtctttcgatacctattcaaggagccttcgcctctggatcccccgccttagttcagcagggcagaacggcggactctaaatccgcatggcacgggttcaaatcccgtaggcgggaccactgcagatccttagcgaaagctaaggatttttttttcggcttatttgctcaagctgcagcgatctcgagctcggtaccctaatacgactcactatagggatggacgaatttgaaatgataaagagaaacacatctgaaattatcagcgaggaagagttaagagaggttttaaaaaaagatgaaaaatctgcttacataggttttgaaccaagtggtaaaatacatttagggcattatctccaaataaaaaagatgattgatttacaaaatgctggatttgatataattatattgttggctgatttagccgcctatttaaaccagaaaggagagttggatgagattagaaaaataggagattataacaaaaaagtttttgaagcaatggggttaaaggcaaaatatgtttatggaagtgaattccagcttgataaggattatacactgaatgtctatagattggctttaaaaactaccttaaaaagagcaagaaggagtatggaacttatagcaagagaggatgaaaatccaaaggttgctgaagttatctatccaataatgcaggttaataccagtcattatttaggcgttgatgttgcagttggagggatggagcagagaaaaatacacatgttagcaagggagcttttaccaaaaaaggttgtttgtattcacaaccctgtcttaacgggtttggatggagaaggaaagatgagttcttcaaaagggaattttatagctgttgatgactctccagaagagattagggctaagataaagaaagcatactgcccagctggagttgttgaaggaaatccaataatggagatagctaaatacttccttgaatatcctttaaccataaaaaggccagaaaaatttggtggagatttgacagttaatagctatgaggagttagagagtttatttaaaaataaggaattgcatccaatgcgtttaaaaaatgctgtagctgaagaacttataaagattttagagccaattagaaagagatta

SEQ ID NO: 102 - DNA, 1038 bp, synthetic construct
  source 1..1038: mol_type = other DNA
  misc_feature 1..1038: note = VHH antibody N15 DNA cassette
caaattcctgtgaagtagctgatttagtacttttcggaggtgtctattcttaccaaatcgtcaagttgtgggtagagtcacctgaatattaattgcaccgcacgggtgatatatgcttatttgctcaagtagttcgaggttaagtgtattttaggtgaacaaatttcagcttcgggtagaagactttcgatgcgcttcagagcttctattgggaaatctgacaccacttgattaaatagcctacccccgaattgggggattggtcattttttgctgtgaaggtagttttgatgcatatgacctgcgtttataaagaaatgtaaacgtgatcagatcgatataaaagaaacagtttgtactcaggtttgaagcattttctccgattcgcctggcaaaaatctcaattgtcgcttacagtttttctcaacgacaggctgctaagctgctagttcggtggcctagtgagtggcgtttacttggataaaagtaatcccatgtcgtgatcagccattttgggttgtttccatagcaatccaaaggtttcgtctttcgatacctattcaaggagccttcgcctctatgtttaacaaccgtatccgcactgcagctctcgctggtgcaatcgcaatctccaccgcagcttccggcgtagctatcccagcattcgctcaggagaccaacccaacccaggtccagttggttgaatccggcggtggccttgtgcagcctggtggctcccttcgcttgtcttgcgcagcttccggcttcaccttctccaacgatgcaatgacctgggtccgtcaggcacctggtaaagcgctcgagtgggtttcctctatcaccctgctcggtggcggtattccatactactctgataccgtgaagggccgcttcaccatctcccgtgacaacaccaaaaacatgctgtacctgcagatgaactctctgaagccagaagataccgcagtctactactgtgctaagggtttcaaatccgactaccctcgcggtcagggcacccaggtgaccgtctcctct

SEQ ID NO: 103 - DNA, 351 bp, synthetic construct
  source 1..351: mol_type = other DNA
  misc_feature 1..351: note = VHH antibody N15 gene
caggtccagttggttgaatccggcggtggccttgtgcagcctggtggctcccttcgcttgtcttgcgcagcttccggcttcaccttctccaacgatgcaatgacctgggtccgtcaggcacctggtaaagcgctcgagtgggtttcctctatcaccctgctcggtggcggtattccatactactctgataccgtgaagggccgcttcaccatctcccgtgacaacaccaaaaacatgctgtacctgcagatgaactctctgaagccagaagataccgcagtctactactgtgctaagggtttcaaatccgactaccctcgcggtcagggcacccaggtgaccgtctcctct

SEQ ID NO: 104 - protein, 117 aa, synthetic construct
  REGION 1..117: note = VHH antibody N15
QVQLVESGGGLVQPGGSLRLSCAASGFTFSNDAMTWVRQAPGKALEWVSSITLLGGGIPYYSDTVKGRFTISRDNTKNMLYLQMNSLKPEDTAVYYCAKGFKSDYPRGQGTQVTVSS

SEQ ID NO: 105 - DNA, 31 bp, synthetic construct
  source 1..31: mol_type = other DNA
  misc_feature 1..31: note = primer
cggtattccatagtactctgataccgtgaag

SEQ ID NO: 106 - DNA, 28 bp, synthetic construct
  source 1..28: mol_type = other DNA
  misc_feature 1..28: note = primer
cagagtactatggaataccgccaccgag

SEQ ID NO: 107 - DNA, 28 bp, synthetic construct
  source 1..28: mol_type = other DNA
  misc_feature 1..28: note = primer
catgctgtagctgcagatgaactctctg

SEQ ID NO: 108 - DNA, 28 bp, synthetic construct
  source 1..28: mol_type = other DNA
  misc_feature 1..28: note = primer
ctgcagctacagcatgtttttggtgttg

SEQ ID NO: 109 - DNA, 31 bp, synthetic construct
  source 1..31: mol_type = other DNA
  misc_feature 1..31: note = primer
cagtctactagtgtgctaagggtttcaaatc

SEQ ID NO: 110 - DNA, 30 bp, synthetic construct
  source 1..30: mol_type = other DNA
  misc_feature 1..30: note = primer
cttagcacactagtagactgcggtatcttc

SEQ ID NO: 111 - DNA, 31 bp, synthetic construct
  source 1..31: mol_type = other DNA
  misc_feature 1..31: note = primer
cggcaactgaaacttcaaggattacgagtac

SEQ ID NO: 112 - DNA, 29 bp, synthetic construct
  source 1..29: mol_type = other DNA
  misc_feature 1..29: note = primer
gaagtttcagttgccggagttgatctggt

SEQ ID NO: 113 - DNA, 1565 bp, Methanosarcina mazei
  source 1..1565: mol_type = genomic DNA
tttacactttatgcttccggctcgtatgttgtgtggaattgtgagcggataacaatttcacacaggaaacagctatgaccatgattacgaattcgagctcggtacccaaattcctgtggaaattaatacgactcactatagggagaccacaacggtttccctctagaaataattttgtttaactttaagaaggagatataccaatggataagaaacctctcaacaccctcatctctgcaaccggtctctggatgtctcgtaccggcaccattcacaagattaaacaccacgaggtctcccgctctaagatctacattgaaatggcatgcggcgatcacttggtggtcaacaactcccgttcctctcgtaccgcacgtgcactgaagcaccacaaataccgcaagacctgcaaacgctgtcgtgtgtccgatgaggacctgaacaagttcctcaccaaagctaacgaagaccagacctctgtgaaggtcaaagttgtgtccgcaccgacccgtaccaagaaagctatgccaaagtccgtcgcacgcgctccaaaacctctggagaacaccgaagcagctcaggcccagccatccgagtctaagttctctccagcgatccctgtgtccacccaggaatccgtttctgtgcctgcctccgtctctacctctatctcctctatttctaccggtgcaaccgcatccgcactggttaagggtaacaccaacccaatcacctctatgtccgctccagtgcaggcttctgcccctgcgttgaccaagtcccagaccgatcgcctggaagtgctgctcaaccctaaggacgaaatctctctcaactccggcaaaccgttccgtgaacttgagtctgaacttttgtcccgccgtaagaaagatctccagcagatctacgcagaagagcgtgagaactacctgggcaagctcgagcgtgaaatcacccgcttcttcgtcgaccgcggtttcctcgaaattaagtccccgatccttattccattggagtacatcgaacgtatgggtattgataacgacaccgagctgtccaagcagatcttccgtgttgataaaaacttctgccttcgccctatgttggcaccgaacctgtacaactacctgcgtaagctcgatcgcgctctgccggacccaatcaagattttcgaaatcggcccatgttaccgcaaggagtccgacggtaaagaacacctcgaagagttcaccatgcttaacttctgccagatgggctccggttgtacccgcgagaacctggaatccatcattaccgatttccttaaccacttgggtatcgatttcaagattgtcggcgactcctgcatggttttcggtgataccctcgacgttatgcacggcgaccttgagttgtcctctgccgtcgttggccctatcccgctcgatcgtgaatggggtatcgacaagccatggattggtgcaggtttcggtcttgagcgtctgctcaaggtgaaacacgatttcaagaacatcaaacgtgctgctcgctctgaatcctactacaacggtatctccaccaacttg

SEQ ID NO: 114 - DNA, 1362 bp, Methanosarcina mazei
  source 1..1362: mol_type = genomic DNA
atggataagaaacctctcaacaccctcatctctgcaaccggtctctggatgtctcgcaccggcaccattcacaaaattaaacaccacgaggtctcccgctctaagatctacattgaaatggcatgcggcgatcacttggtggtcaacaactcccgttcctctcgtaccgcacgtgcactgaagcaccacaaataccgcaagacctgcaaacgctgtcgtgtgtccgatgaggacctgaacaagttcctcaccaaagctaacgaagaccagacctctgtgaaggtcaaagttgtgtccgcaccgacccgtaccaagaaagctatgccaaagtccgtcgcacgcgctccaaaacctctggagaacaccgaagcagctcaggcccagccatccgagtctaagttctctccagcgatccctgtgtccacccaggaatccgtttctgtgcctgcctccgtctctacctctatctcctctatttctaccggtgcaaccgcatccgcactggttaagggtaacaccaacccaatcacctctatgtccgctccagtgcaggcttctgcccctgcgttgaccaagtcccagaccgatcgcctggaagtgctgctcaaccctaaggacgaaatctctctcaactccggcaaaccgttccgtgaacttgagtctgaacttttgtcccgccgtaagaaagatctccagcagatctacgcagaagagcgtgagaactacctgggcaagctcgagcgtgaaatcacccgcttcttcgtcgaccgcggtttcctcgaaattaagtccccgatccttattccattggagtacatcgaacgtatgggtattgataacgacaccgagctgtccaagcagatcttccgtgttgataaaaacttctgccttcgccctatgttggcaccgaacctgtacaactacctgcgtaagctcgatcgcgctctgccggacccaatcaagattttcgaaatcggcccatgttaccgcaaggagtccgacggtaaagaacacctcgaagagttcaccatgcttaacttctgccagatgggctccggttgtacccgcgagaacctggaatccatcattaccgatttccttaaccacttgggtatcgatttcaagattgtcggcgactcctgcatggttttcggtgataccctcgacgttatgcacggcgaccttgagttgtcctctgccgtcgttggccctatcccgctcgatcgtgaatggggtatcgacaagccatggattggtgcaggtttcggtcttgagcgtctgctcaaggtgaaacacgatttcaagaacattaaacgcgcagcacgctctgagtcctactacaacggtatctccaccaacttg

SEQ ID NO: 115 - protein, 454 aa, Methanosarcina mazei
MDKKPLNTLISATGLWMSRTGTIHKIKHHEVSRSKIYIEMACGDHLVVNNSRSSRTARALKHHKYRKTCKRCRVSDEDLNKFLTKANEDQTSVKVKVVSAPTRTKKAMPKSVARAPKPLENTEAAQAQPSESKFSPAIPVSTQESVSVPASVSTSISSISTGATASALVKGNTNPITSMSAPVQASAPALTKSQTDRLEVLLNPKDEISLNSGKPFRELESELLSRRKKDLQQIYAEERENYLGKLEREITRFFVDRGFLEIKSPILIPLEYIERMGIDNDTELSKQIFRVDKNFCLRPMLAPNLYNYLRKLDRALPDPIKIFEIGPCYRKESDGKEHLEEFTMLNFCQMGSGCTRENLESIITDFLNHLGIDFKIVGDSCMVFGDTLDVMHGDLELSSAVVGPIPLDREWGIDKPWIGAGFGLERLLKVKHDFKNIKRAARSESYYNGISTNL

SEQ ID NO: 116 - DNA, 72 bp, Methanosarcina mazei
  source 1..72: mol_type = genomic DNA
ggaaacctgatcatgtagatcgaatggactctaaatccgttcagccgggttagattcccggggtttccgcca

SEQ ID NO: 117 - DNA, 72 bp, Methanosarcina mazei
  source 1..72: mol_type = genomic DNA
ggaaacctgatcatgtagatcgaatggacttcaaatccgttcagccgggttagattcccggggtttccgcca

SEQ ID NO: 118 - DNA, 72 bp, Methanosarcina mazei; identical to SEQ ID NO: 116
  source 1..72: mol_type = genomic DNA

SEQ ID NO: 119 - RNA, 72 nt, Methanosarcina mazei
  source 1..72: mol_type = tRNA
ggaaacctgatcatgtagatcgaatggactctaaatccgttcagccgggttagattcccggggtttccgcca

SEQ ID NO: 120 - DNA, 72 bp, Methanosarcina mazei; identical to SEQ ID NO: 117
  source 1..72: mol_type = genomic DNA

SEQ ID NO: 121 - RNA, 72 nt, Methanosarcina mazei
  source 1..72: mol_type = tRNA
ggaaacctgatcatgtagatcgaatggacttcaaatccgttcagccgggttagattcccggggtttccgcca

SEQ ID NO: 122 - DNA, 562 bp, synthetic construct
  source 1..562: mol_type = other DNA
  misc_feature 1..562: note = VHH antibody 9g8 DNA cassette
taatacgactcactataggggaattgtgagcggataacaattcccctctagaaataattttgtttaactttaagaaggagatatacatatgaaatacctgctgccgaccgctgctgctggtctgctgctcctcgctgcccagccggcgatggccgaagtgcagctggtggaaagcggtggcggcctggttcaggcgggtggtagtctgcgcttatcttgtgcggcgtctggtcgtacattttcttcatatgccatgggctggtttcgccaagctccaggcaaagaacgcgagtttgtggtggctattaactggtcttctggcagcacctattatgcggattccgtcaaaggccgcttcacgattagccgtgataacgccaagaatacgatgtacctccagatgaacagcctgaaaccggaagataccgccgtctactattgcgctgcaggctatcagatcaacagcggcaactataactttaaagattacgagtacgactattggggtcaaggcactcaggttaccgtgtcgtcggcactcgagcaccaccaccaccaccac

SEQ ID NO: 123 - DNA, 1036 bp, Methanocaldococcus jannaschii
  source 1..1036: mol_type = genomic DNA
ggtacccaaattcctgtggaaattaatacgactcactatagggagaccacaacggtttccctctagaaataattttgtttaactttaagaaggagatataccaatggatgaatttgaaatgattaagcgtaacaccagcgaaattatctcggaagaagaactgcgtgaagtcctgaaaaaggatgaaaaatcggccaccatcggctttgaaccgagcggtaaaattcatctgggccactatctgcagatcaaaaagatgattgatctgcaaaacgcaggtttcgacattatcattctgctggcggatctgcatgcctatctgaaccagaaaggtgaactggacgaaatccgtaagatcggcgattacaacaagaaggtgtttgaagcgatgggtctgaaagccaagtatgtttacggctctaacttccaactggataaagactataccctgaatgtttaccgtctggcactgaaaaccacgctgaagcgcgctcgtcgctccatggaactgattgcgcgcgaagacgaaaacccgaaagttgcggaagtcatctatccgattatgcaagtgaatccgctgcactaccaaggcgttgatgtcgctgtgggcggtatggaacagcgtaaaatccatatgctggcgcgcgaactgctgccgaaaaaggtggtttgcattcacaacccggtcctgacgggtctggatggcgaaggtaaaatgagctctagtaagggcaattttatcgccgtggatgacagcccggaagaaatccgtgcaaagattaaaaaggcatactgtccggctggcgtcgtggaaggtaatccgatcatggaaattgccaaatattttctggaatacccgctgaccattaaacgcccggaaaagttcggcggtgacctgacggttaactcctacgaagaactggaatcactgttcaaaaataaggaactgcatccgatggatctgaaaaacgccgtcgccgaagaactgattaaaatcctggaaccgatccgcaaacgcctgtaagggccctctaga

SEQ ID NO: 124 - DNA, 1124 bp, Methanocaldococcus jannaschii
  source 1..1124: mol_type = genomic DNA
ggtacccggggatccaccggcgcctgactgcagatccttagcgaaagctaaggatttttttttcggcttatttgctcaagctgcagcgatctcgagctcggtacccgaaattaatacgactcactatagggagaccacaacggtttccctctagaaataattttgtttaactttaagaaggagatataccaatggatgaatttgaaatgattaagcgtaacaccagcgaaattatctcggaagaagaactgcgtgaagtcctgaaaaaggatgaaaaatcggccaccatcggctttgaaccgagcggtaaaattcatctgggccactatctgcagatcaaaaagatgattgatctgcaaaacgcaggtttcgacattatcattctgctggcggatctgcatgcctatctgaaccagaaaggtgaactggacgaaatccgtaagatcggcgattacaacaagaaggtgtttgaagcgatgggtctgaaagccaagtatgtttacggctctaacttccaactggataaagactataccctgaatgtttaccgtctggcactgaaaaccacgctgaagcgcgctcgtcgctccatggaactgattgcgcgcgaagacgaaaacccgaaagttgcggaagtcatctatccgattatgcaagtgaatccgctgcactaccaaggcgttgatgtcgctgtgggcggtatggaacagcgtaaaatccatatgctggcgcgcgaactgctgccgaaaaaggtggtttgcattcacaacccggtcctgacgggtctggatggcgaaggtaaaatgagctctagtaagggcaattttatcgccgtggatgacagcccggaagaaatccgtgcaaagattaaaaaggcatactgtccggctggcgtcgtggaaggtaatccgatcatggaaattgccaaatattttctggaatacccgctgaccattaaacgcccggaaaagttcggcggtgacctgacggttaactcctacgaagaactggaatcactgttcaaaaataaggaactgcatccgatggatctgaaaaacgccgtcgccgaagaactgattaaaatcctggaaccgatccgcaaacgcctgtaagggccctctaga

SEQ ID NO: 125 - DNA, 844 bp, synthetic construct
  source 1..844: mol_type = other DNA
  misc_feature 1..844: note = WT-aMD4dY-PA22 DNA cassette
caaattcctgtgaagtagctgatttagtacttttcggaggtgtctattcttaccaaatcgtcaagttgtgggtagagtcacctgaatattaattgcaccgcacgggtgatatatgcttatttgctcaagtagttcgaggttaagtgtattttaggtgaacaaatttcagcttcgggtagaagactttcgatgcgcttcagagcttctattgggaaatctgacaccacttgattaaatagcctacccccgaattgggggattggtcattttttgctgtgaaggtagttttgatgcatatgacctgcgtttataaagaaatgtaaacgtgatcagatcgatataaaagaaacagtttgtactcaggtttgaagcattttctccgattcgcctggcaaaaatctcaattgtcgcttacagtttttctcaacgacaggctgctaagctgctagttcggtggcctagtgagtggcgtttacttggataaaagtaatcccatgtcgtgatcagccattttgggttgtttccatagcaatccaaaggtttcgtctttcgatacctattcaaggagccttcgatgtttaacaaccgtatccgcactgcagctctcgctggtgcaatcgcaatctccaccgcagcttccggcgtagctatcccagcattcgctgcagagacctgccgtcagttcaaccgtcgcacccacgaagtttggaatctggactgtggcgcagcccccgcagcacccgctcccgcagcacccgcagctccagcaccagcagccccagcagcaccaggctgccgccagttcaaccgtcgcacccacgaagtgtggaatttggattgttaa

SEQ ID NO: 126 - DNA, 180 bp, synthetic construct
  source 1..180: mol_type = other DNA
  misc_feature 1..180: note = WT-aMD4dY-PA22 gene
gcagagacctgccgtcagttcaaccgtcgcacccacgaagtttggaatctggactgtggcgcagcccccgcagcacccgctcccgcagcacccgcagctccagcaccagcagccccagcagcaccaggctgccgccagttcaaccgtcgcacccacgaagtgtggaatttggattgttaa

SEQ ID NO: 127 - protein, 59 aa, synthetic construct
  REGION 1..59: note = WT-aMD4dY-PA22
AETCRQFNRRTHEVWNLDCGAAPAAPAPAAPAAPAPAAPAAPGCRQFNRRTHEVWNLDC

SEQ ID NO: 128 - DNA, 183 bp, synthetic construct
  source 1..183: mol_type = other DNA
  misc_feature 1..183: note = N-AzF-aMD4dY-PA22 gene
gcagagacctagtgccgtcagttcaaccgtcgcacccacgaagtttggaatctggactgtggcgcagcccccgcagcacccgctcccgcagcacccgcagctccagcaccagcagccccagcagcaccaggctgccgccagttcaaccgtcgcacccacgaagtgtggaatttggattgttaa

SEQ ID NO: 129 - protein, 60 aa, synthetic construct
  REGION 1..60: note = N-AzF-aMD4dY-PA22
  VARIANT 4: note = X is AzF
AETXCRQFNRRTHEVWNLDCGAAPAAPAPAAPAAPAPAAPAAPGCRQFNRRTHEVWNLDC

SEQ ID NO: 130 - DNA, 183 bp, synthetic construct
  source 1..183: mol_type = other DNA
  misc_feature 1..183: note = L1-AzF-aMD4dY-PA22 gene
gcagagacctgccgtcagttcaaccgtcgcacccacgaagtttggaatctggactgtggcgcagcccccgcagcacccgctcccgcagcacccgcataggctccagcaccagcagccccagcagcaccaggctgccgccagttcaaccgtcgcacccacgaagtgtggaatttggattgttaa

SEQ ID NO: 131 - protein, 60 aa, synthetic construct
  REGION 1..60: note = L1-AzF-aMD4dY-PA22
  VARIANT 33: note = X is AzF
AETCRQFNRRTHEVWNLDCGAAPAAPAPAAPAXAPAPAAPAAPGCRQFNRRTHEVWNLDC

SEQ ID NO: 132 - DNA, 180 bp, synthetic construct
  source 1..180: mol_type = other DNA
  misc_feature 1..180: note = L2-AzF-aMD4dY-PA22 gene
gcagagacctgccgtcagttcaaccgtcgcacccacgaagtttggaatctggactgtggcgcagcccccgcagcacccgctcccgcagcataggcagctccagcaccagcagccccagcagcaccaggctgccgccagttcaaccgtcgcacccacgaagtgtggaatttggattgttaa

SEQ ID NO: 133 - protein, 59 aa, synthetic construct
  REGION 1..59: note = L2-AzF-aMD4dY-PA22
  VARIANT 31: note = X is AzF
AETCRQFNRRTHEVWNLDCGAAPAAPAPAAXAAPAPAAPAAPGCRQFNRRTHEVWNLDC

SEQ ID NO: 134 - DNA, 862 bp, synthetic construct
  source 1..862: mol_type = other DNA
  misc_feature 1..862: note = WT-EPO-PA22 DNA cassette
caaattcctgtgaagtagctgatttagtacttttcggaggtgtctattcttaccaaatcgtcaagttgtgggtagagtcacctgaatattaattgcaccgcacgggtgatatatgcttatttgctcaagtagttcgaggttaagtgtattttaggtgaacaaatttcagcttcgggtagaagactttcgatgcgcttcagagcttctattgggaaatctgacaccacttgattaaatagcctacccccgaattgggggattggtcattttttgctgtgaaggtagttttgatgcatatgacctgcgtttataaagaaatgtaaacgtgatcagatcgatataaaagaaacagtttgtactcaggtttgaagcattttctccgattcgcctggcaaaaatctcaattgtcgcttacagtttttctcaacgacaggctgctaagctgctagttcggtggcctagtgagtggcgtttacttggataaaagtaatcccatgtcgtgatcagccattttgggttgtttccatagcaatccaaaggtttcgtctttcgatacctattcaaggagccttcgatgtttaacaaccgtatccgcactgcagctctcgctggtgcaatcgcaatctccaccgcagcttccggcgtagctatcccagcattcgctgcagagaccggcggcctttacgcttgtcacatgggtccaatgacctgggtctgtcaacctctccgtggtgcagccccggcagcccccgctccagccgcaccagcagccccagccccagctgcaccagccgctccaggcggcctctacgcctgccacatgggtcctatgacctgggtgtgccaaccacttcgcggctaa

SEQ ID NO: 135 - DNA, 198 bp, synthetic construct
  source 1..198: mol_type = other DNA
  misc_feature 1..198: note = WT-EPO-PA22 gene
gcagagaccggcggcctttacgcttgtcacatgggtccaatgacctgggtctgtcaacctctccgtggtgcagccccggcagcccccgctccagccgcaccagcagccccagccccagctgcaccagccgctccaggcggcctctacgcctgccacatgggtcctatgacctgggtgtgccaaccacttcgcggctaa

SEQ ID NO: 136 - protein, 65 aa, synthetic construct
  REGION 1..65: note = WT-EPO-PA22
AETGGLYACHMGPMTWVCQPLRGAAPAAPAPAAPAAPAPAAPAAPGGLYACHMGPMTWVCQPLRG

SEQ ID NO: 137 - DNA, 201 bp, synthetic construct
  source 1..201: mol_type = other DNA
  misc_feature 1..201: note = N-AzF-EPO-PA22 gene
gcagagacctagggcggcctttacgcttgtcacatgggtccaatgacctgggtctgtcaacctctccgtggtgcagccccggcagcccccgctccagccgcaccagcagccccagccccagctgcaccagccgctccaggcggcctctacgcctgccacatgggtcctatgacctgggtgtgccaaccacttcgcggctaa

SEQ ID NO: 138 - protein, 66 aa, synthetic construct
  REGION 1..66: note = N-AzF-EPO-PA22
  VARIANT 4: note = X is AzF
AETXGGLYACHMGPMTWVCQPLRGAAPAAPAPAAPAAPAPAAPAAPGGLYACHMGPMTWVCQPLRG

SEQ ID NO: 139 - DNA, 201 bp, synthetic construct
  source 1..201: mol_type = other DNA
  misc_feature 1..201: note = L1-AzF-EPO-PA22 gene
gcagagaccggcggcctttacgcttgtcacatgggtccaatgacctgggtctgtcaacctctccgtggtgcagccccggcagcccccgctccagccgcaccagcataggccccagccccagctgcaccagccgctccaggcggcctctacgcctgccacatgggtcctatgacctgggtgtgccaaccacttcgcggctaa

SEQ ID NO: 140 - protein, 66 aa, synthetic construct
  REGION 1..66: note = L1-AzF-EPO-PA22
  VARIANT 36: note = X is AzF
AETGGLYACHMGPMTWVCQPLRGAAPAAPAPAAPAXAPAPAAPAAPGGLYACHMGPMTWVCQPLRG

SEQ ID NO: 141 - DNA, 198 bp, synthetic construct
  source 1..198: mol_type = other DNA
  misc_feature 1..198: note = L2-AzF-EPO-PA22 gene
gcagagaccggcggcctttacgcttgtcacatgggtccaatgacctgggtctgtcaacctctccgtggtgcagccccggcagcccccgctccagccgcataggcagccccagccccagctgcaccagccgctccaggcggcctctacgcctgccacatgggtcctatgacctgggtgtgccaaccacttcgcggctaa

SEQ ID NO: 142 - protein, 65 aa, synthetic construct
  REGION 1..65: note = L2-AzF-EPO-PA22
  VARIANT 34: note = X is AzF
AETGGLYACHMGPMTWVCQPLRGAAPAAPAPAAXAAPAPAAPAAPGGLYACHMGPMTWVCQPLRG